European Patent Specification EP 3 773 626 B1, published January 28, 2026. Title: USE OF HISTONE MODIFIERS TO REPROGRAM EFFECTOR T CELLS. Applicant: Board of Regents, The University of Texas System YEE, CASSIAN WANG, JUNMEI. The sequence listing filed with the application follows.

SEQUENCE LISTING (13 sequences)

SEQ ID NO: 1 - protein, 162 aa, Homo sapiens
MRSSPGNMERIVICLMVIFLGTLVHKSSSQGQDRHMIRMRQLIDIVDQLKNYVNDLVPEFLPAPEDVETNCEWSAFSCFQKAQLKSANTGNNERIINVSIKKLKRKPPSTNAGRRQKHRLTCPSCDSYEKKPPKEFLERFKSLLQKMIHQHLSSRTHGSEDS

SEQ ID NO: 2 - DNA, 21 bp, Artificial Sequence
  Primer
ctcacacttcgggttcctcgg

SEQ ID NO: 3 - DNA, 21 bp, Artificial Sequence
  Primer
gactccaccaaccaccaccag

SEQ ID NO: 4 - DNA, 20 bp, Artificial Sequence
  Primer
atggaacgatgacgcctgcc

SEQ ID NO: 5 - DNA, 20 bp, Artificial Sequence
  Primer
ggcctccaaaggctcacact

SEQ ID NO: 6 - DNA, 20 bp, Artificial Sequence
  Primer
cacacccgtcacacatccca

SEQ ID NO: 7 - DNA, 22 bp, Artificial Sequence
  Primer
tgggaaaaccagccaagaggtg

SEQ ID NO: 8 - DNA, 20 bp, Artificial Sequence
  Primer
tgcagctatacccaggctgg

SEQ ID NO: 9 - DNA, 19 bp, Artificial Sequence
  Primer
cctcgaccgcctcttcttc

SEQ ID NO: 10 - DNA, 21 bp, Artificial Sequence
  Primer
tctgctggatttcaagcaccc

SEQ ID NO: 11 - DNA, 21 bp, Artificial Sequence
  Primer
gactgcagcatttcacacagg

SEQ ID NO: 12 - DNA, 20 bp, Artificial Sequence
  Primer
tgcttgcacgtagaatgggt

SEQ ID NO: 13 - DNA, 20 bp, Artificial Sequence
  Primer
ggatggggacaggttgtgtc